European Patent Specification EP 3 485 014 B1, published September 6, 2023. Title: Improved PNA Probe. Applicant: DestiNA Genomica S.L. Ilyine, Hugh A Diaz-Mochon, Juan J Pernagallo, Salvatore J Chavez, Mavys T Fara, Mario A. The sequence listing filed with the application follows.

SEQUENCE LISTING (27 sequences)

SEQ ID NO: 1 - DNA, 17 bp, Artificial Sequence
  DGL-12DAV-6neg
  modified_base (2)..(2): Gamma modified thymine
  misc_feature (2)..(2): n is a, c, g, or t
  modified_base (5)..(5): Gamma modified guanine
  misc_feature (5)..(5): n is a, c, g, or t
  modified_base (8)..(8): Gamma modified adenine
  misc_feature (8)..(10): n is a, c, g, or t
  modified_base (9)..(9): Abasic position
  modified_base (10)..(10): Gamma modified cytosine
  modified_base (13)..(13): Gamma modified cytosine
  misc_feature (13)..(13): n is a, c, g, or t
  misc_feature (15)..(15): n is a, c, g, or t
  modified_base (16)..(16): Gamma modified cytosine
cnacnccnnnagntnaa

SEQ ID NO: 2 - DNA, 18 bp, Artificial Sequence
  DGL-12SRC-6neg
  modified_base (2)..(2): Gamma modified thymine
  misc_feature (2)..(2): n is a, c, g, or t
  modified_base (6)..(6): Gamma modified cytosine
  misc_feature (6)..(6): n is a, c, g, or t
  modified_base (9)..(9): Gamma modified cytosine
  misc_feature (9)..(11): n is a, c, g, or t
  modified_base (10)..(10): Abasic position
  modified_base (11)..(11): Gamma modified adenine
  modified_base (14)..(14): Gamma modified thymine
  modified_base (17)..(17): Gamma modified adenine
  misc_feature (17)..(17): n is a, c, g, or t
cnacgncannngctccna

SEQ ID NO: 3 - DNA, 18 bp, Artificial Sequence
  DGL-13SRC-6neg
  modified_base (3)..(3): Gamma modified guanine
  misc_feature (3)..(3): n is a, c, g, or t
  modified_base (6)..(6): Gamma modified thymine
  misc_feature (6)..(6): n is a, c, g, or t
  modified_base (10)..(10): Gamma modified cytosine
  misc_feature (10)..(12): n is a, c, g, or t
  modified_base (11)..(11): Abasic position
  modified_base (12)..(12): Gamma modified adenine
  modified_base (15)..(15): Gamma modified adenine
  misc_feature (15)..(15): n is a, c, g, or t
  modified_base (17)..(17): Gamma modified cytosine
  misc_feature (17)..(17): n is a, c, g, or t
ttnccnacgnnnccngnt

SEQ ID NO: 4 - DNA, 18 bp, Artificial Sequence
  DGL-13DAV-6neg
  modified_base (3)..(3): Gamma modified guanine
  misc_feature (3)..(3): n is a, c, g, or t
  modified_base (6)..(6): Gamma modified thymine
  misc_feature (6)..(6): n is a, c, g, or t
  modified_base (9)..(9): Gamma modified guanine
  misc_feature (9)..(11): n is a, c, g, or t
  modified_base (10)..(10): Abasic position
  modified_base (11)..(11): Gamma modified cytosine
  modified_base (14)..(14): Gamma modified cytosine
  misc_feature (14)..(14): n is a, c, g, or t
  modified_base (17)..(17): Gamma modified cytosine
  misc_feature (17)..(17): n is a, c, g, or t
ttnccnacnnnacnagnt

SEQ ID NO: 5 - DNA, 22 bp, Artificial Sequence
  KWT DNA
ttggagctggtggcgtaggcaa

SEQ ID NO: 6 - DNA, 18 bp, Artificial Sequence
  DNA K125
ttggagctagtggcgtag

SEQ ID NO: 7 - DNA, 18 bp, Artificial Sequence
  DGL-12DAV
  misc_feature (9)..(9): n is a, c, g, or t
ctacgccancagctccaa

SEQ ID NO: 8 - DNA, 18 bp, Artificial Sequence
  DGL-12SRC
  modified_base (10)..(10): Gamma modified abasic position
  misc_feature (10)..(10): n is a, c, g, or t
ctacgccacnagctccaa

SEQ ID NO: 9 - DNA, 18 bp, Artificial Sequence
  DGL-13SRC
  modified_base (11)..(11): Gamma modified abasic position
  misc_feature (11)..(11): n is a, c, g, or t
ttgcctacgcnaccagct

SEQ ID NO: 10 - DNA, 18 bp, Artificial Sequence
  DGL-13DAV
  modified_base (10)..(10): Gamma modified abasic position
  misc_feature (10)..(10): n is a, c, g, or t
ttgcctacgncaccagct

SEQ ID NO: 11 - DNA, 18 bp, Artificial Sequence
  DGL-12DAV-3CC
  modified_base (8)..(8): Gamma modified adenine
  misc_feature (8)..(10): n is a, c, g, or t
  modified_base (9)..(9): Gamma modified abasic position
  modified_base (10)..(10): Gamma modified cytosine
ctacgccnnnagctccaa

SEQ ID NO: 12 - DNA, 18 bp, Artificial Sequence
  DGL-12SRC-3CC
  modified_base (9)..(9): Gamma modified cytosine
  misc_feature (9)..(11): n is a, c, g, or t
  modified_base (10)..(10): Gamma modified abasic position
  modified_base (11)..(11): Gamma modified adenine
ctacgccannngctccaa

SEQ ID NO: 13 - DNA, 18 bp, Artificial Sequence
  DGL-12DAV-3RCC
  modified_base (7)..(7): Gamma modified cytosine
  misc_feature (7)..(7): n is a, c, g, or t
  modified_base (9)..(9): Gamma modified abasic position
  misc_feature (9)..(9): n is a, c, g, or t
  modified_base (11)..(11): Gamma modified adenine
  misc_feature (11)..(11): n is a, c, g, or t
ctacgcnancngctccaa

SEQ ID NO: 14 - DNA, 18 bp, Artificial Sequence
  DGL-12SRC-3RCC
  modified_base (8)..(8): Gamma modified adenine
  misc_feature (8)..(8): n is a, c, g, or t
  modified_base (10)..(10): Gamma modified abasic position
  misc_feature (10)..(10): n is a, c, g, or t
  modified_base (12)..(12): Gamma modified guanine
  misc_feature (12)..(12): n is a, c, g, or t
ctacgccncnanctccaa

SEQ ID NO: 15 - DNA, 18 bp, Artificial Sequence
  DGL-13SRC-3RCC
  modified_base (9)..(9): Gamma modified guanine
  misc_feature (9)..(9): n is a, c, g, or t
  modified_base (11)..(11): Gamma modified abasic position
  misc_feature (11)..(11): n is a, c, g, or t
  modified_base (13)..(13): Gamma modified cytosine
  misc_feature (13)..(13): n is a, c, g, or t
ttgcctacncnancagct

SEQ ID NO: 16 - DNA, 18 bp, Artificial Sequence
  DGL-13DAV-3RCC
  modified_base (8)..(8): Gamma modified cytosine
  misc_feature (8)..(8): n is a, c, g, or t
  modified_base (10)..(10): Gamma modified abasic position
  misc_feature (10)..(10): n is a, c, g, or t
  modified_base (12)..(12): Gamma modified adenine
  misc_feature (12)..(12): n is a, c, g, or t
ttgcctangncnccagct

SEQ ID NO: 17 - RNA, 22 nt, Homo sapiens
uggagugugacaaugguguuug

SEQ ID NO: 18 - DNA, 18 bp, Artificial Sequence
  DGL122_1.2
  modified_base (3)..(3): gamma modified cytosine
  misc_feature (3)..(3): n is a, c, g, or t
  modified_base (5)..(5): gamma modified cytosine
  misc_feature (5)..(6): n is a, c, g, or t
  modified_base (6)..(6): Abasic position
  modified_base (8)..(8): gamma modified thymine
  misc_feature (8)..(8): n is a, c, g, or t
  modified_base (11)..(11): gamma modified thymine
  misc_feature (11)..(11): n is a, c, g, or t
  modified_base (14)..(14): gamma modified cytosine
  misc_feature (14)..(14): n is a, c, g, or t
  modified_base (16)..(16): gamma modified cytosine
  misc_feature (16)..(16): n is a, c, g, or t
aanannantgncanantc

SEQ ID NO: 19 - DNA, 17 bp, Artificial Sequence
  DGL122_3.0
  modified_base (7)..(7): Abasic position
  misc_feature (7)..(7): n is a, c, g, or t
caaacancattgtcaca

SEQ ID NO: 20 - DNA, 17 bp, Artificial Sequence
  DGL122_5.0
  modified_base (11)..(11): Abasic position
  misc_feature (11)..(11): n is a, c, g, or t
accattgtcanactcca

SEQ ID NO: 21 - DNA, 18 bp, Artificial Sequence
  DGL122_4.0
  modified_base (10)..(10): Abasic position
  misc_feature (10)..(10): n is a, c, g, or t
caccattgtnacactcca

SEQ ID NO: 22 - DNA, 18 bp, Artificial Sequence
  DGL122_4.1
  modified_base (6)..(6): Gamma modified thymine
  misc_feature (6)..(6): n is a, c, g, or t
  modified_base (9)..(9): Gamma modified thymine
  misc_feature (9)..(10): n is a, c, g, or t
  modified_base (10)..(10): Abasic position
  modified_base (15)..(15): Gamma modified thymine
  misc_feature (15)..(15): n is a, c, g, or t
caccantgnnacacncca

SEQ ID NO: 23 - DNA, 18 bp, Artificial Sequence
  DGL122_4.2
  modified_base (6)..(6): Gamma modified thymine
  misc_feature (6)..(6): n is a, c, g, or t
  modified_base (9)..(9): Gamma modified thymine
  misc_feature (9)..(10): n is a, c, g, or t
  modified_base (10)..(10): Gamma modified abasic position
  modified_base (15)..(15): Gamma modified thymine
  misc_feature (15)..(15): n is a, c, g, or t
caccantgnnacacncca

SEQ ID NO: 24 - DNA, 19 bp, Artificial Sequence
  DGL21_2.0
  modified_base (7)..(7): Gamma modified thymine
  misc_feature (7)..(7): n is a, c, g, or t
  modified_base (9)..(9): Abasic position
  misc_feature (9)..(9): n is a, c, g, or t
  modified_base (11)..(11): Gamma modified thymine
  misc_feature (11)..(11): n is a, c, g, or t
tcaacancngnctcagata

SEQ ID NO: 25 - DNA, 17 bp, Artificial Sequence
  DGL21_3.0
  modified_base (8)..(8): Gamma modified thymine
  misc_feature (8)..(8): n is a, c, g, or t
  modified_base (10)..(10): Abasic position
  misc_feature (10)..(10): n is a, c, g, or t
  modified_base (15)..(15): Gamma modified cytosine
  misc_feature (15)..(15): n is a, c, g, or t
atcagtcngntaagnta

SEQ ID NO: 26 - DNA, 19 bp, Artificial Sequence
  DGL21_6.0
  modified_base (6)..(6): Gamma modified thymine
  misc_feature (6)..(6): n is a, c, g, or t
  modified_base (8)..(8): Gamma modified abasic position
  misc_feature (8)..(8): n is a, c, g, or t
  modified_base (10)..(10): Gamma modified thymine
  misc_feature (10)..(10): n is a, c, g, or t
caacancngnctgataagc

SEQ ID NO: 27 - RNA, 22 nt, Homo sapiens
uagcuuaucagacugauguuga